European Patent Application EP 4 467 652 A1, published November 27, 2024. Title: 1,4-Butanediol producing microorganism and method for producing 1,4-butanediol using the same. Applicant: DAESANG CORPORATION. The sequence listing filed with the application follows.

SEQUENCE LISTING (63 sequences)

SEQ ID NO: 1 - DNA, 1683 bp, Pseudomonas putida
  source 1..1683: mol_type = genomic DNA
atgaacaagaagaaccgccaccccgccgacggcaagaagccgatcaccattttcggcccggacttcccttttgctttcgacgactggctggaacacccggcaggcctgggcagcattccggctgagcgccatggggaagaggtggccattgtcggtgccggtatcgccggcctggtagcggcctacgagctgatgaagctgggcctcaagccggtggtgtacgaggcttccaagctgggcggccggctgcgctcgcaagccttcaatggcactgacgggatcgttgccgagctgggtggcatgcgcttcccggtgtcgtccaccgccttctaccactacgtcgacaagctgggcctggagaccaagcccttccccaacccgctgaccccggcttcgggcagcacggtgatcgacctggaaggccagacctactacgccgagaagcccaccgacctgccgcaactgtttcatgaggtagccgacgcttgggccgatgctctggagagcggtgcgcagttcgccgatatccagcaggccatccgcgaccgtgatgtaccgcgcctgaaggaactctggaacaagctggtgccactgtgggacgaccgcaccttctacgacttcgtcgccacctcgcgctcttttgccaagctgagcttccagcaccgcgaagtgttcggccaggtcggtttcggcaccggcggttgggactcggacttccccaactcgatgctggaaatcttccgcgtggtgatgaccaactgcgacgaccaccagcacctggtggtcgggggcgtggaacaagtgccacaaggcatctggcgcgacgtaccggaacgctgcgtgcattggccagagggcaccagcctgagcacgctgcatggcggcgcaccgcgtaccggggtcaagcgcattgcccgcgccgccgatggccgcctggcggtcaccgacaactggggcgatacccgccactacagcgcagtactcgccacctgccagacctggttgctgaccacccagatcgactgcgaggaatcgctgttctcgcaaaagatgtggatggccctggaccgtacccgctacatgcagtcgtcgaaaaccttcgtcatggtcgaccgcccgttctggaaggacaaggacccggaaaccggccgtgacctgctgagcatgaccctcaccgaccgcctcacccgcggcacttacctgttcgacaacggcaacgacaagcccggggtgatctgcctgtcgtactcgtggatgagcgacgcgctgaagatgctgccgcacccggtggaaaagcgcgtacaactggccctggatgcgctgaagaagatctacccgaagaccgatatcgccgggcacatcatcggcgacccgatcacggtttcctgggaggccgacccgtacttcctcggcgccttcaaaggcgcgcttccgggccattaccgctacaaccagcgcatgtacgcgcacttcatgcagcaggacatgccggcggagcagcgcggtatcttcattgccggtgacgacgtgtcatggacccccgcctgggttgaaggcgcggtgcagacgtcgctgaatgcggtgtggggtatcatgaaccactttggtggccacacccaccccgacaaccccggcccgggcgatgtgttcaacgaaatcggcccgatcgccctggcggattga

SEQ ID NO: 2 - protein, 560 aa, Pseudomonas putida
MNKKNRHPADGKKPITIFGPDFPFAFDDWLEHPAGLGSIPAERHGEEVAIVGAGIAGLVAAYELMKLGLKPVVYEASKLGGRLRSQAFNGTDGIVAELGGMRFPVSSTAFYHYVDKLGLETKPFPNPLTPASGSTVIDLEGQTYYAEKPTDLPQLFHEVADAWADALESGAQFADIQQAIRDRDVPRLKELWNKLVPLWDDRTFYDFVATSRSFAKLSFQHREVFGQVGFGTGGWDSDFPNSMLEIFRVVMTNCDDHQHLVVGGVEQVPQGIWRDVPERCVHWPEGTSLSTLHGGAPRTGVKRIARAADGRLAVTDNWGDTRHYSAVLATCQTWLLTTQIDCEESLFSQKMWMALDRTRYMQSSKTFVMVDRPFWKDKDPETGRDLLSMTLTDRLTRGTYLFDNGNDKPGVICLSYSWMSDALKMLPHPVEKRVQLALDALKKIYPKTDIAGHIIGDPITVSWEADPYFLGAFKGALPGHYRYNQRMYAHFMQQDMPAEQRGIFIAGDDVSWTPAWVEGAVQTSLNAVWGIMNHFGGHTHPDNPGPGDVFNEIGPIALAD

SEQ ID NO: 3 - DNA, 795 bp, Pseudomonas putida
  source 1..795: mol_type = genomic DNA
atgcgcatcgctctgtaccagggcgcacccaagccactggatgtgcccggcaacctgcaacggctgcgccaccaggcgcagttggcagccgaccgcggcgcacagttgctggtgtgcccggagatgttcctgtccggctacaacatcggcctggcccaggtcgagcgcctggccgaggccgccgatggcccggcagccatgacggtggtggagattgcccaggcgcaccgtatcgccattgtctatggctacccggagcgcggcgatgacggggcgatctacaacagcgtgcagctgatcgatgcgcatggccgcagcctgagcaattaccgcaagacccacctgttcggtgaactggaccgctcgatgttcagccctggtgcggaccacttcccggtggtggaactggaaggctggaaggttggcctgctgatctgctacgacatcgagttcccggagaacgcccgacgcctggcgctggacggcgccgagctgatcctggtgccgacggcgaacatgacgccgtacgactttacctgccaggtgaccgtgagggcacgggcgcaggaaaaccagtgctacctggtatatgccaactactgcggcgcggaagacgagatcgagtattgcgggcagagcagcatcatcggcccggatggcagcttgctggccatggccgggcgggatgagtgccagttgttggcagagctcgagcatgagcgggtggtgcaggggcgcagggcgtttccctacctgaccgatttgcgccaggagctgcacctgcgtaaaggctga

SEQ ID NO: 4 - protein, 264 aa, Pseudomonas putida
MRIALYQGAPKPLDVPGNLQRLRHQAQLAADRGAQLLVCPEMFLSGYNIGLAQVERLAEAADGPAAMTVVEIAQAHRIAIVYGYPERGDDGAIYNSVQLIDAHGRSLSNYRKTHLFGELDRSMFSPGADHFPVVELEGWKVGLLICYDIEFPENARRLALDGAELILVPTANMTPYDFTCQVTVRARAQENQCYLVYANYCGAEDEIEYCGQSSIIGPDGSLLAMAGRDECQLLAELEHERVVQGRRAFPYLTDLRQELHLRKG

SEQ ID NO: 5 - DNA, 1347 bp, Corynebacterium glutamicum
  source 1..1347: mol_type = genomic DNA
gtggaagatctctcataccgcatcccgcagtcgcgcaccgtggccgagcaggtgccagggccgaagtcgaaagcgctggatgagcgtcgacaagcagcagtagcacgagcacttgcaccgggtctgcctggatacgtggtggacgcagacggtggcatcttggctgacgcggacggcaaccgtttcatcgacctggcctccggcatcgccgtgaccacggtcggcggatccaacgcggccgtcgcgaaagccgtcggcgccgcagctgcccgcttcacccacacctgcttcatggtctcaccttatgaaacttacgtggccatggcggagagactcaacgccttgactccaggcgatcacgacaagaagagcgcgctgtttaactctggcgccgaagccgtggaaaacgccgtcaaggtggcacgcgcctacaccggcaagggcgcggtcgtggtgttcgacaacgcgtaccacggacggaccaacctcaccatggcgatgaccgcgaagaaccgcccatacaagtccggattcggaccactagccgcagacgtctaccgtgcaccaatgtcttacccactgcgcgacggactgtccggcccggaagccgcagagcgcgcgatctccgtgatcgaatcccaggtcggagccgaaaacctcgcctgcgtggtcattgaaccgatccagggcgaaggcggattcatcgtccccgcaccaggattcctcgcagccatttccacctggtgccgcgagaacgacgtggtgttcatcgccgatgaaatccaatctggcttcctgcgcaccggcgactggttcgccagcgacgcagaaggtgtgatccccgacgtcatcaccaccgcaaaaggcatcgccggcggcatgccactatccgcagtgaccggccgcgcagaaatcatggacgcacccggccccggcgcgctcggcggaacctacggcggaaaccccgttgcttgcgccgcggcacttgcagccattgaagtgatggaacaagccgaccttaagacccgcgcgcaagaaatcgagaccatcatccgcgatgaattcgcgcagctgagtgccttcccggaggtcgccgaaatccgcggccgcggagcaatgatggccattgagcttatcgacgctaccggccgcccgaacgcagctttaaccgccgcagtggctgcgcgcgcaaaagctgaaggtgtgctgctgctgacttgcggcaccgatggcaacgtcatccgcctgctgccaccactggtcattgcagaggacactctccgtgatggtcttcaggtgttagtcgcagccctagagcgcgaaaccgcgcaccagaaggtgggctaa

SEQ ID NO: 6 - protein, 448 aa, Corynebacterium glutamicum
VEDLSYRIPQSRTVAEQVPGPKSKALDERRQAAVARALAPGLPGYVVDADGGILADADGNRFIDLASGIAVTTVGGSNAAVAKAVGAAAARFTHTCFMVSPYETYVAMAERLNALTPGDHDKKSALFNSGAEAVENAVKVARAYTGKGAVVVFDNAYHGRTNLTMAMTAKNRPYKSGFGPLAADVYRAPMSYPLRDGLSGPEAAERAISVIESQVGAENLACVVIEPIQGEGGFIVPAPGFLAAISTWCRENDVVFIADEIQSGFLRTGDWFASDAEGVIPDVITTAKGIAGGMPLSAVTGRAEIMDAPGPGALGGTYGGNPVACAAALAAIEVMEQADLKTRAQEIETIIRDEFAQLSAFPEVAEIRGRGAMMAIELIDATGRPNAALTAAVAARAKAEGVLLLTCGTDGNVIRLLPPLVIAEDTLRDGLQVLVAALERETAHQKVG

SEQ ID NO: 7 - DNA, 1050 bp, Escherichia coli
  source 1..1050: mol_type = genomic DNA
atgaagatcaaagctgttggtgcatattccgctaaacaaccacttgaaccgatggatatcacccggcgtgaaccgggaccgaatgatgtcaaaatcgaaatcgcttactgtggcgtttgccattccgatctccaccaggtccgttccgagtgggcggggacggtttacccctgcgtgccgggtcatgaaattgtggggcgtgtggtagccgttggtgatcaggtagaaaaatatgcgccgggcgatctggtcggtgtcggctgcattgtcgacagttgtaaacattgcgaagagtgtgaagacgggttggaaaactactgtgatcacatgaccggcacctataactcgccgacgccggacgaaccgggccatactctgggcggctactcacaacagatcgtcgttcatgagcgatatgttctgcgtattcgtcacccgcaagagcagctggcggcggtggctcctttgttgtgtgcagggatcaccacgtattcgccgctacgtcactggcaggccgggccgggtaaaaaagtgggcgtggtcggcatcggcggtctgggacatatggggattaagctggcccacgcgatgggggcacatgtggtggcatttaccacttctgaggcaaaacgcgaagcggcaaaagccctgggggccgatgaagttgttaactcacgcaatgccgatgagatggcggctcatctgaagagtttcgatttcattttgaatacagtagctgcgccacataatctcgacgattttaccaccttgctgaagcgtgatggcaccatgacgctggttggtgcgcctgcgacaccgcataaatcgccggaagttttcaacctgatcatgaaacgccgtgcgatagccggttctatgattggcggcattccagaaactcaggagatgctcgatttttgcgccgaacatggcatcgtggctgatatagagatgattcgggccgatcaaattaatgaagcctatgagcgaatgctgcgcggtgatgtgaaatatcgttttgttatcgataatcgcacactaacagactga

SEQ ID NO: 8 - protein, 349 aa, Escherichia coli
MKIKAVGAYSAKQPLEPMDITRREPGPNDVKIEIAYCGVCHSDLHQVRSEWAGTVYPCVPGHEIVGRVVAVGDQVEKYAPGDLVGVGCIVDSCKHCEECEDGLENYCDHMTGTYNSPTPDEPGHTLGGYSQQIVVHERYVLRIRHPQEQLAAVAPLLCAGITTYSPLRHWQAGPGKKVGVVGIGGLGHMGIKLAHAMGAHVVAFTTSEAKREAAKALGADEVVNSRNADEMAAHLKSFDFILNTVAAPHNLDDFTTLLKRDGTMTLVGAPATPHKSPEVFNLIMKRRAIAGSMIGGIPETQEMLDFCAEHGIVADIEMIRADQINEAYERMLRGDVKYRFVIDNRTLTD

SEQ ID NO: 9 - DNA, 3537 bp, Mycobacterium abscessus
  source 1..3537: mol_type = genomic DNA
atgactgaaacgatctccacagcggctgtccccactacggatctcgaagagcaggtgaagcgacgcatcgagcaggtcgtgtccaacgatccgcagctggcggcgcttctcccggaagattcggtcaccgaggcggtcaacgagcccgatctaccgctggtcgaggtgatcaggcgactgctggagggctacggtgaccgcccggcactcggccagcgcgccttcgagttcgtcaccggggacgacggtgcgaccgtgatcgcgctgaagcccgaatacaccaccgtctcctaccgcgagttgtgggaacgtgccgaggctatcgctgccgcgtggcacgagcagggcatccgtgacggcgacttcgtcgctcagttgggtttcaccagcacggacttcgcgtcgctcgacgtcgcgggattgcgtctgggcaccgtctcggtgcccctgcagacgggcgcgtcgctgcagcagcgcaacgcgattctcgaagagacccggcccgcagtctttgccgcgagtatcgaataccttgatgccgccgtcgattcggtgcttgcgaccccctcggtgcgactcctctcggttttcgactatcacgcggaggtcgacagccagcgcgaagcgctggaggctgtgcgggcccggcttgagagtgccggccggacgatcgtcgtcgaggccctggcggaggctctcgcgcgggggcgggacctgcccgccgcgccgctgcccagtgcagatcccgatgccttgcgtctgctcatctacacctccggcagcaccggtacccccaagggcgccatgtatccgcaatggctggtcgccaacttgtggcagaagaagtggctcaccgacgatgtgattccgtccataggcgtgaacttcatgcccatgagccacctggcgggtcgcctcactctcatgggcaccctttccggtggcggaaccgcctactacatcgcttcgagcgatctttcgactttcttcgaggacatcgcgctcatccgcccctccgaagtgctcttcgtgccgcgtgtggtggagatggtgttccagcgttttcaggcagaattggaccggtcccttgccccgggtgagagcaactccgagatcgcggagcgaatcaaggtccgcatccgggaacaggacttcggcgggcgtgtgctcagtgctggctccgggtcggccccgttgtctcctgagatgacggagttcatggagtcgctgctgcaggtgccgttgcgcgacgggtatgggtccaccgaggccggtggtgtgtggcgtgacggagtcctgcagcgtccgcccgtcaccgactacaagctggttgacgttccggaactcggatacttcaccacagattcgccgcatccccgtggcgagctgcggttgaagtcggagacgatgttccccggctactacaagcgcccggagaccactgccgatgtcttcgatgacgaggggtactacaagaccggtgacgtggtcgccgagctcgggccggatcacctcaagtacctcgaccgcgtcaagaacgtcctcaagctcgcgcagggagagtttgtcgcggtgtcaaagctggaggccgcttacaccggcagcccgctggtccggcagatctttgtgtacgggaacagtgaacgctcgttcctgctggctgtcgtggtcccgacacccgaagtccttgagcggtacgcagattcgccagatgcgctcaagcccttgatccaggattcgctgcagcaggtcgccaaggacgcggagctgcaatcctatgagataccgcgcgacttcatcgttgagacggtgccgttcaccgtcgagtccggattgctatcggacgcgcgaaagctgctgcgccccaagctgaaggatcactacggagagaggctggaggcgctgtacgccgaactggcggaaagccagaatgagcggctgcgccagttggccagggaggcagccacgcgcccggtcctggagacggtgaccgatgcggccgccgcgctgctgggcgcatcgtcctcggatctggctcctgatgtgcgattcatcgacctcggtggcgactcactgtcggcgctgtcgtactccgagctgctgcgcgacatctttgaggtggacgttccggtgggcgtcatcaacagcgtcgccaacgaccttgccgcgatcgcccggcacatcgaggcgcagcggaccggcgccgctacgcagccgacctttgcgtcggtccacggcaaggacgcgacggtcatcaccgccggtgaactcaccctcgacaagttcttggacgagtcactgttgaaagcggccaaggacgttcagccggcaacggccgatgtcaagaccgttctagtgaccggcggcaacggctggttgggtcgttggctggtgctcgattggctggagcggttggcacccaatggtggcaaggtctacgccctcattcgtggcgccgatgccgaagcagcccgggcacggttggacgccgtgtacgaatcgggtgatcccaagctgtccgcgcattatcgtcagctggcgcaacagagtctggaagttatcgccggcgatttcggcgaccaggatctcggtctatcccaggaagtttggcagaagctggccaaggacgtggacctgatcgtgcactccggtgccttggtgaaccacgtgctgccgtacagccagttgttcggtccgaatgtggcgggtaccgccgagatcatcaagctggcaatttcggagcggctcaagccggtcacctacctgtcgacggtgggcatcgccgaccagattccggtgacggagttcgaggaagactccgatgttcgtgtgatgtcggccgagcgccagatcaatgacggctacgcgaacggatacggcaactcaaaatgggccggcgaggtgctgttgcgggaggctcatgacctagcggggctgccggtgcgtgtgttccgctccgacatgatcctggcgcacagtgactaccacggacagctcaacgtcaccgacgtgttcacccggagcatccagagtctgctgctcaccggtgttgcaccggccagcttctatgaattggatgccgacggcaatcggcagcgcgctcactatgacggtgtgcccggcgatttcaccgccgcatcgatcaccgccatcggcggtgtgaacgtggtagacggttaccgcagcttcgacgtgttcaacccgcaccatgacggtgtctcgatggataccttcgtcgactggctgatcgacgcaggctacaagatcgcgcggatcgacgattacgaccagtggctcgcccggttcgagctggccctcaagggattgcccgagcagcagcggcaacagtcggtgttgccacttctcaagatgtacgagaagccgcaaccggcgatcgacggaagtgcacttccgaccgcagaattcagtcgcgccgtgcacgaggcgaaggtcggagacagcggtgagataccgcacgtcaccaaggagctgatcctcaagtacgccagcgatattcagctgttgggcctggtgtag

SEQ ID NO: 10 - protein, 1178 aa, Mycobacterium abscessus
MTETISTAAVPTTDLEEQVKRRIEQVVSNDPQLAALLPEDSVTEAVNEPDLPLVEVIRRLLEGYGDRPALGQRAFEFVTGDDGATVIALKPEYTTVSYRELWERAEAIAAAWHEQGIRDGDFVAQLGFTSTDFASLDVAGLRLGTVSVPLQTGASLQQRNAILEETRPAVFAASIEYLDAAVDSVLATPSVRLLSVFDYHAEVDSQREALEAVRARLESAGRTIVVEALAEALARGRDLPAAPLPSADPDALRLLIYTSGSTGTPKGAMYPQWLVANLWQKKWLTDDVIPSIGVNFMPMSHLAGRLTLMGTLSGGGTAYYIASSDLSTFFEDIALIRPSEVLFVPRVVEMVFQRFQAELDRSLAPGESNSEIAERIKVRIREQDFGGRVLSAGSGSAPLSPEMTEFMESLLQVPLRDGYGSTEAGGVWRDGVLQRPPVTDYKLVDVPELGYFTTDSPHPRGELRLKSETMFPGYYKRPETTADVFDDEGYYKTGDVVAELGPDHLKYLDRVKNVLKLAQGEFVAVSKLEAAYTGSPLVRQIFVYGNSERSFLLAVVVPTPEVLERYADSPDALKPLIQDSLQQVAKDAELQSYEIPRDFIVETVPFTVESGLLSDARKLLRPKLKDHYGERLEALYAELAESQNERLRQLAREAATRPVLETVTDAAAALLGASSSDLAPDVRFIDLGGDSLSALSYSELLRDIFEVDVPVGVINSVANDLAAIARHIEAQRTGAATQPTFASVHGKDATVITAGELTLDKFLDESLLKAAKDVQPATADVKTVLVTGGNGWLGRWLVLDWLERLAPNGGKVYALIRGADAEAARARLDAVYESGDPKLSAHYRQLAQQSLEVIAGDFGDQDLGLSQEVWQKLAKDVDLIVHSGALVNHVLPYSQLFGPNVAGTAEIIKLAISERLKPVTYLSTVGIADQIPVTEFEEDSDVRVMSAERQINDGYANGYGNSKWAGEVLLREAHDLAGLPVRVFRSDMILAHSDYHGQLNVTDVFTRSIQSLLLTGVAPASFYELDADGNRQRAHYDGVPGDFTAASITAIGGVNVVDGYRSFDVFNPHHDGVSMDTFVDWLIDAGYKIARIDDYDQWLARFELALKGLPEQQRQQSVLPLLKMYEKPQPAIDGSALPTAEFSRAVHEAKVGDSGEIPHVTKELILKYASDIQLLGLV

SEQ ID NO: 11 - DNA, 675 bp, Bacillus subtilis
  source 1..675: mol_type = genomic DNA
atgaagatttacggaatttatatggaccgcccgctttcacaggaagaaaatgaacggttcatgactttcatatcacctgaaaaacgggagaaatgccggagattttatcataaagaagatgctcaccgcaccctgctgggagatgtgctcgttcgctcagtcataagcaggcagtatcagttggacaaatccgatatccgctttagcacgcaggaatacgggaagccgtgcatccctgatcttcccgacgctcatttcaacatttctcactccggccgctgggtcattggtgcgtttgattcacagccgatcggcatagatatcgaaaaaacgaaaccgatcagccttgagatcgccaagcgcttcttttcaaaaacagagtacagcgaccttttagcaaaagacaaggacgagcagacagactatttttatcatctatggtcaatgaaagaaagctttatcaaacaggaaggcaaaggcttatcgcttccgcttgattccttttcagtgcgcctgcatcaggacggacaagtatccattgagcttccggacagccattccccatgctatatcaaaacgtatgaggtcgatcccggctacaaaatggctgtatgcgccgcacaccctgatttccccgaggatatcacaatggtctcgtacgaagagcttttataa

SEQ ID NO: 12 - protein, 224 aa, Bacillus subtilis
MKIYGIYMDRPLSQEENERFMTFISPEKREKCRRFYHKEDAHRTLLGDVLVRSVISRQYQLDKSDIRFSTQEYGKPCIPDLPDAHFNISHSGRWVIGAFDSQPIGIDIEKTKPISLEIAKRFFSKTEYSDLLAKDKDEQTDYFYHLWSMKESFIKQEGKGLSLPLDSFSVRLHQDGQVSIELPDSHSPCYIKTYEVDPGYKMAVCAAHPDFPEDITMVSYEELL

SEQ ID NO: 13 - DNA, 68 bp, synthetic construct
  source 1..68: mol_type = other DNA
ggatcctttcacacaggaaacagaccatgcaccatcatcaccatcacatgaacaagaagaaccgccac

SEQ ID NO: 14 - DNA, 25 bp, synthetic construct
  source 1..25: mol_type = other DNA
aagctttcagcctttacgcaggtgc

SEQ ID NO: 15 - DNA, 1683 bp, synthetic construct
  source 1..1683: mol_type = other DNA
atgaacaagaataaccgccatcctgcagatgggaaaaaaccgatcacaatttttggcccggacttcccttttgcctttgatgattggctggaacacccagctggactgggtagcattccagcagcgcgacatggtgaggaagttgctatcgtgggtgccggcattgccgggctggtggcggcctacgaactgatgaagctgggcttaaaaccggtggtctatgaagcgtcgaaaatgggtgggcggctgagatcacaggcattcaatggcacggatggaataatagccgagctgggaggaatgcgctttccggtgtcttccacggcgttctatcactacgttgataagttaggcctagaaacgaagccttttcctaaccccctcactcctgcctcacgttcaacggtaatagatctggaagggcagacctattacgcggaaaaagcagccgatttgccagccctttttcaggaagttaccgatgcctgggctgacgccctggaaagcggtgcgcgctttggtgatatccagcaagcaattagggatcgtgatgtgcctcgcttgaaagaactgtggaacaccctggttccactgtgggacgaccgtactttttatgattttgtcgccacatccaaagcttttgccaaactgtcttttcaacaccgcgaggttttcggccaggttggctttggcaccggtggttgggattcggatttccccaattcgatgctggaaatcttccgtgtagttatgaccaattgcgacgaccatcaacatctggtggttggcggcgtcgagcaagtaccgcagggtatctggaggcatgtgccagagcgttgtgcgcattggcccgaaggtacatcactgagttctctgcacggcggtgctccgagaaccggcgtgaaacgcattgcccgggcaagtgacggccgactggcagtcacagacaactggggcgactgcagacattacgcagccgtattaacgacatgtcagagttggctgctgaccactcagatcgactgtgaagaaagcttgttttcacagaagatgtggatggctctagatagaactcgttatatgcaatcttcgaaaacctttgtaatggtcgaccggccgttttggaaagacaaagacccagaaactggtcgcgacctgatgagcatgacgcttactgaccgcctgacccgtggcacctatttattcgataatggcgacgacaaaccaggagtaatctgcttaagttatgcatggatgagcgatgctctgaaaatgctcccccatccggttgaaaaacgtgtccaactggcattagatgcattgaaaaagatctacccgaaaacggatattgccgggcatattattggcgaccctattacaatttcttgggaagctgatcctcacttcctcggtgcattcaaaggcgcgctgccgggccactatcgctataaccagcggatgtatgcgcattttatgcaggcacagatgccagtagagcagcgtggaattttcattgctggcgacgacgtgtcgtggaccccggcatgggtcgaaggcgcggtgcaaacatcgctcaatgcagtgtggggtataatgaatcattttggtggcaaaacccatgctgacaatccgggccctggagatgtgttcgatgagatcggccaaatagcgctggcggactaa

SEQ ID NO: 16 - DNA, 1683 bp, synthetic construct
  source 1..1683: mol_type = other DNA
atgaacaagaataaccgccatcctgcagatgggaaaaaaccgatcacaatttttggcccggacttcccttttgcctttgatgattggctggaacacccagctggactgggtagcattccagcagcgcgacatggtgaggaagttgctatcgtgggtgccggcattgccgggctggtggcggcctacgaactgatgaagctgggcttaaaaccggtggtctatgaagcgtcgaaaatgggtgggcggctgagatcacaggcattcaatggcacggatggaataatagccgagctgggaggaatgcgctttccggtgtcttccacggcgttctatcactacgttgataagttaggcctagaaacgaagccttttcctaaccccctcactcctgcctcacgttcaacggtaatagatctggaagggcagacctattacgcggaaaaagcagccgatttgccagccctttttcaggaagttaccgatgcctgggctgacgccctggaaagcggtgcgcgctttggtgatatccagcaagcaattagggatcgtgatgtgcctcgcttgaaagaactgtggaacaccctggttccactgtgggacgaccgtactttttatgattttgtcgccacatccaaagcttttgccaaactgtcttttcaacaccgcgaggttttcggccaggttggctttggcaccggtggttgggattcggatttccccaattcgatgctggaaatcttccgtgtagttatgaccaatattgacgaccatcaacatctggtggttggcggcgtcgagcaagtaccgcagggtatctggaggcatgtgccagagcgttgtgcgcattggcccgaaggtacatcactgagttctctgcacggcggtgctccgagaaccggcgtgaaacgcattgcccgggcaagtgacggccgactggcagtcacagacaactggggcgactgcagacattacgcagccgtattaacgacatgtcagagttggctgctgaccactcagatcgactgtgaagaaagcttgttttcacagaagatgtggatggctctagatagaactcgttatatgcaatcttcgaaaacctttgtaatggtcgaccggccgttttggaaagacaaagacccagaaactggtcgcgacctgatgagcatgacgcttactgaccgcctgacccgtggcacctatttattcgataatggcgacgacaaaccaggagtaatctgcttaagttatgcatggatgagcgatgctctgaaaatgctcccccatccggttgaaaaacgtgtccaactggcattagatgcattgaaaaagatctacccgaaaacggatattgccgggcatattattggcgaccctattacaatttcttgggaagctgatcctcacttcctcggtgcattcaaaggcgcgctgccgggccactatcgctataaccagcggatgtatgcgcattttatgcaggcacagatgccagtagagcagcgtggaattttcattgctggcgacgacgtgtcgtggaccccggcatgggtcgaaggcgcggtgcaaacatcgctcaatgcagtgtggggtataatgaatcattttggtggcaaaacccatgctgacaatccgggccctggagatgtgttcgatgagatcggccaaatagcgctggcggactaa

SEQ ID NO: 17 - DNA, 1683 bp, synthetic construct
  source 1..1683: mol_type = other DNA
atgaacaagaataaccgccatcctgcagatgggaaaaaaccgatcacaatttttggcccggacttcccttttgcctttgatgattggctggaacacccagctggactgggtagcattccagcagcgcgacatggtgaggaagttgctatcgtgggtgccggcattgccgggctggtggcggcctacgaactgatgaagctgggcttaaaaccggtggtctatgaagcgtcgaaaatgggtgggcggctgagatcacaggcattcaatggcacggatggaataatagccgagctgggaggaatgcgctttccggtgtcttccacggcgttctatcactacgttgataagttaggcctagaaacgaagccttttcctaaccccctcactcctgcctcacgttcaacggtaatagatctggaagggcagacctattacgcggaaaaagcagccgatttgccagccctttttcaggaagttaccgatgcctgggctgacgccctggaaagcggtgcgcgctttggtgatatccagcaagcaattagggatcgtgatgtgcctcgcttgaaagaactgtggaacaccctggttccactgtgggacgaccgtactttttatgattttgtcgccacatccaaagcttttgccaaactgtcttttcaacaccgcgaggttttcggccaggttggctttggcaccggtggttgggattcggatttccccaattcgatgctggaaatcttccgtgtagttatgaccaatcttgacgaccatcaacatctggtggttggcggcgtcgagcaagtaccgcagggtatctggaggcatgtgccagagcgttgtgcgcattggcccgaaggtacatcactgagttctctgcacggcggtgctccgagaaccggcgtgaaacgcattgcccgggcaagtgacggccgactggcagtcacagacaactggggcgactgcagacattacgcagccgtattaacgacatgtcagagttggctgctgaccactcagatcgactgtgaagaaagcttgttttcacagaagatgtggatggctctagatagaactcgttatatgcaatcttcgaaaacctttgtaatggtcgaccggccgttttggaaagacaaagacccagaaactggtcgcgacctgatgagcatgacgcttactgaccgcctgacccgtggcacctatttattcgataatggcgacgacaaaccaggagtaatctgcttaagttatgcatggatgagcgatgctctgaaaatgctcccccatccggttgaaaaacgtgtccaactggcattagatgcattgaaaaagatctacccgaaaacggatattgccgggcatattattggcgaccctattacaatttcttgggaagctgatcctcacttcctcggtgcattcaaaggcgcgctgccgggccactatcgctataaccagcggatgtatgcgcattttatgcaggcacagatgccagtagagcagcgtggaattttcattgctggcgacgacgtgtcgtggaccccggcatgggtcgaaggcgcggtgcaaacatcgctcaatgcagtgtggggtataatgaatcattttggtggcaaaacccatgctgacaatccgggccctggagatgtgttcgatgagatcggccaaatagcgctggcggactaa

SEQ ID NO: 18 - DNA, 25 bp, synthetic construct
  source 1..25: mol_type = other DNA
gaattcatgaacaagaataaccgcc

SEQ ID NO: 19 - DNA, 27 bp, synthetic construct
  source 1..27: mol_type = other DNA
ggtaccttagtccgccagcgctatttg

SEQ ID NO: 20 - DNA, 36 bp, synthetic construct
  source 1..36: mol_type = other DNA
tgattacgccaagcttggtacgtaccttatccgcgc

SEQ ID NO: 21 - DNA, 40 bp, synthetic construct
  source 1..40: mol_type = other DNA
ccttcggatctaaacgatctggtgacctcttctctgaaac

SEQ ID NO: 22 - DNA, 40 bp, synthetic construct
  source 1..40: mol_type = other DNA
gtttcagagaagaggtcaccagatcgtttagatccgaagg

SEQ ID NO: 23 - DNA, 39 bp, synthetic construct
  source 1..39: mol_type = other DNA
ggcggttcttcttgttcattgtatgtcctcctggacttc

SEQ ID NO: 24 - DNA, 40 bp, synthetic construct
  source 1..40: mol_type = other DNA
gaagtccaggaggacatacaatgaacaagaagaaccgcca

SEQ ID NO: 25 - DNA, 80 bp, synthetic construct
  source 1..80: mol_type = other DNA
cgacaaacaacagataaaacgaaaggcccagtctttcgactgagcctttcgttttatttgtcaatccgccagggcgatcg

SEQ ID NO: 26 - DNA, 80 bp, synthetic construct
  source 1..80: mol_type = other DNA
gactgggcctttcgttttatctgttgtttgtcggtgaacgctctcctgagtaggacaaatagatcgtttagatccgaagg

SEQ ID NO: 27 - DNA, 40 bp, synthetic construct
  source 1..40: mol_type = other DNA
tggtacagagcgatgcgcattgtatgtcctcctggacttc

SEQ ID NO: 28 - DNA, 40 bp, synthetic construct
  source 1..40: mol_type = other DNA
gaagtccaggaggacatacaatgcgcatcgctctgtacca

SEQ ID NO: 29 - DNA, 40 bp, synthetic construct
  source 1..40: mol_type = other DNA
ggaggggttttacttagatttcagcctttacgcaggtgca

SEQ ID NO: 30 - DNA, 40 bp, synthetic construct
  source 1..40: mol_type = other DNA
tgcacctgcgtaaaggctgaaatctaagtaaaacccctcc

SEQ ID NO: 31 - DNA, 34 bp, synthetic construct
  source 1..34: mol_type = other DNA
ccggggatcctctagaatggtgggatccatcgcg

SEQ ID NO: 32 - DNA, 34 bp, synthetic construct
  source 1..34: mol_type = other DNA
tgattacgccaagctagatgctcattgaccgggg

SEQ ID NO: 33 - DNA, 40 bp, synthetic construct
  source 1..40: mol_type = other DNA
ccttcggatctaaacgatcttgctacggcagctccaatcc

SEQ ID NO: 34 - DNA, 40 bp, synthetic construct
  source 1..40: mol_type = other DNA
ggattggagctgccgtagcaagatcgtttagatccgaagg

SEQ ID NO: 35 - DNA, 40 bp, synthetic construct
  source 1..40: mol_type = other DNA
ccaacagctttgatcttcattgtatgtcctcctggacttc

SEQ ID NO: 36 - DNA, 40 bp, synthetic construct
  source 1..40: mol_type = other DNA
gaagtccaggaggacatacaatgaagatcaaagctgttgg

SEQ ID NO: 37 - DNA, 40 bp, synthetic construct
  source 1..40: mol_type = other DNA
aattggcagctaagtagggtggttttactgctactttgat

SEQ ID NO: 38 - DNA, 40 bp, synthetic construct
  source 1..40: mol_type = other DNA
agtagcagtaaaaccaccctacttagctgccaattattcc

SEQ ID NO: 39 - DNA, 40 bp, synthetic construct
  source 1..40: mol_type = other DNA
cggtatgagagatcttccacgggtaaaaaatcctttcgta

SEQ ID NO: 40 - DNA, 40 bp, synthetic construct
  source 1..40: mol_type = other DNA
tacgaaaggattttttacccgtggaagatctctcataccg

SEQ ID NO: 41 - DNA, 40 bp, synthetic construct
  source 1..40: mol_type = other DNA
accacatagctggcttcgtcttagcccaccttctggtgcg

SEQ ID NO: 42 - DNA, 40 bp, synthetic construct
  source 1..40: mol_type = other DNA
cgcaccagaaggtgggctaagacgaagccagctatgtggt

SEQ ID NO: 43 - DNA, 33 bp, synthetic construct
  source 1..33: mol_type = other DNA
ccggggatcctctagcaagcaccggtcgattgc

SEQ ID NO: 44 - DNA, 40 bp, synthetic construct
  source 1..40: mol_type = other DNA
gaccatgattacgccaagctcgacgcagaaggtgtgatcc

SEQ ID NO: 45 - DNA, 80 bp, synthetic construct
  source 1..80: mol_type = other DNA
cgacaaacaacagataaaacgaaaggcccagtctttcgactgagcctttcgttttatttgtttagcccaccttctggtgc

SEQ ID NO: 46 - DNA, 80 bp, synthetic construct
  source 1..80: mol_type = other DNA
gactgggcctttcgttttatctgttgtttgtcggtgaacgctctcctgagtaggacaaataccctacttagctgccaatt

SEQ ID NO: 47 - DNA, 40 bp, synthetic construct
  source 1..40: mol_type = other DNA
taaattccgtaaatcttcatgggtaaaaaatcctttcgta

SEQ ID NO: 48 - DNA, 40 bp, synthetic construct
  source 1..40: mol_type = other DNA
aaggattttttacccatgaagatttacggaatttatatgg

SEQ ID NO: 49 - DNA, 39 bp, synthetic construct
  source 1..39: mol_type = other DNA
tcacggcaaagcgaggtacttataaaagctcttcgtacg

SEQ ID NO: 50 - DNA, 40 bp, synthetic construct
  source 1..40: mol_type = other DNA
cgtacgaagagcttttataagtacctcgctttgccgtgac

SEQ ID NO: 51 - DNA, 40 bp, synthetic construct
  source 1..40: mol_type = other DNA
ggtacccggggatcctctagcgaagcttgccgtgtgcagg

SEQ ID NO: 52 - DNA, 40 bp, synthetic construct
  source 1..40: mol_type = other DNA
tgattacgccaagctaataagtttgcccccgatcttcaca

SEQ ID NO: 53 - DNA, 40 bp, synthetic construct
  source 1..40: mol_type = other DNA
aattggcagctaagtagggtgattgctgcgacagtctcat

SEQ ID NO: 54 - DNA, 40 bp, synthetic construct
  source 1..40: mol_type = other DNA
atgagactgtcgcagcaatcaccctacttagctgccaatt

SEQ ID NO: 55 - DNA, 40 bp, synthetic construct
  source 1..40: mol_type = other DNA
ggagatcgtttcagtcatgggtaaaaaatcctttcgtagg

SEQ ID NO: 56 - DNA, 40 bp, synthetic construct
  source 1..40: mol_type = other DNA
aaggattttttacccatgactgaaacgatctccacagcgg

SEQ ID NO: 57 - DNA, 40 bp, synthetic construct
  source 1..40: mol_type = other DNA
tgttcttgccacgttcctgctacaccaggcccaacagctg

SEQ ID NO: 58 - DNA, 40 bp, synthetic construct
  source 1..40: mol_type = other DNA
agctgttgggcctggtgtagcaggaacgtggcaagaacat

SEQ ID NO: 59 - DNA, 33 bp, synthetic construct
  source 1..33: mol_type = other DNA
ccggggatcctctagggcgaccagccggaaaga

SEQ ID NO: 60 - DNA, 40 bp, synthetic construct
  source 1..40: mol_type = other DNA
tggcggttattcttgttcattgtatgtcctcctggacttc

SEQ ID NO: 61 - DNA, 40 bp, synthetic construct
  source 1..40: mol_type = other DNA
gaagtccaggaggacatacaatgaacaagaataaccgcca

SEQ ID NO: 62 - DNA, 37 bp, synthetic construct
  source 1..37: mol_type = other DNA
ggttttacttagattttagtccgccagcgctatttgg

SEQ ID NO: 63 - DNA, 41 bp, synthetic construct
  source 1..41: mol_type = other DNA
caaatagcgctggcggactaaaatctaagtaaaacccctcc